European Patent Application EP 4 494 656 A1, published January 22, 2025. Title: ORGANIC CYTOTOXIN OLIGOMERS AND USES THEREOF AS A PAYLOAD IN ANTIBODY-DRUG CONJUGATES. Applicant: SIMRIS BIOLOGICS GMBH. The sequence listing filed with the application follows.

SEQUENCE LISTING (16 sequences)

SEQ ID NO: 1 - protein, 8 aa, Amanita sp.
  CROSSLNK 1..8: note = peptide bond
  CROSSLNK 2..6: note = sulfoxide bridge
  VARIANT 1: note = Ile, Hydroxyisoleucine or Dihydroxyisoleucine
  VARIANT 2: note = Trp or Hydroxytryptophane
  VARIANT 7: note = Asn or Asp
  VARIANT 8: note = Pro or 4Hyp
IWGIGCJP

SEQ ID NO: 2 - protein, 7 aa, synthetic construct
  CROSSLNK 1..7: note = peptide bond
  SITE 1: note = D-Ala
  SITE 2: note = Propargyltyrosine
  SITE 3: note = D-Asp
  SITE 5: note = 3-amino-9-methoxy-2,6,8-trimethyl-10-phenyl-deca-4,6-dienoic acid
  SITE 6: note = D-Glu
  SITE 7: note = N-methyldehydroalanine
AYDRXEX

SEQ ID NO: 3 - protein, 7 aa, synthetic construct
  CROSSLNK 1..7: note = peptide bond
  SITE 1: note = D-Ala
  SITE 2: note = Propargyllysine
  SITE 3: note = D-Asp
  SITE 5: note = 3-amino-9-methoxy-2,6,8-trimethyl-10-phenyl-deca-4,6-dienoic acid
  SITE 6: note = D-Glu
  SITE 7: note = N-methyldehydroalanine
AKDRXEX

SEQ ID NO: 4 - protein, 7 aa, synthetic construct
  CROSSLNK 1..7: note = peptide bond
  SITE 1: note = D-Ala
  SITE 2: note = Azidophenylalanine
  SITE 3: note = D-Asp
  SITE 5: note = 3-amino-9-methoxy-2,6,8-trimethyl-10-phenyl-deca-4,6-dienoic acid
  SITE 6: note = D-Glu
  SITE 7: note = N-methyldehydroalanine
AFDRXEX

SEQ ID NO: 5 - protein, 7 aa, synthetic construct
  CROSSLNK 1..7: note = peptide bond
  SITE 1: note = D-Ala
  SITE 2: note = Azidolysine
  SITE 3: note = D-Asp
  SITE 5: note = 3-amino-9-methoxy-2,6,8-trimethyl-10-phenyl-deca-4,6-dienoic acid
  SITE 6: note = D-Glu
  SITE 7: note = N-methyldehydroalanine
AKDRXEX

SEQ ID NO: 6 - protein, 7 aa, synthetic construct
  SITE 1: note = D-Ala
  SITE 2: note = Azidonorvaline
  SITE 3: note = D-Asp
  SITE 5: note = 3-amino-9-methoxy-2,6,8-trimethyl-10-phenyl-deca-4,6-dienoic acid
  SITE 6: note = D-Glu
  SITE 7: note = N-methyldehydroalanine
  CROSSLNK 1..7: note = Peptide bond
AXDRXEX

SEQ ID NO: 7 - protein, 7 aa, synthetic construct
  SITE 1: note = D-Ala
  SITE 3: note = D-Asp
  SITE 4: note = Propargyltyrosine
  SITE 5: note = 3-amino-9-methoxy-2,6,8-trimethyl-10-phenyl-deca-4,6-dienoic acid
  SITE 6: note = D-Glu
  SITE 7: note = N-methyldehydroalanine
  CROSSLNK 1..7: note = Peptide bond
ALDYXEX

SEQ ID NO: 8 - protein, 7 aa, synthetic construct
  SITE 1: note = D-Ala
  SITE 3: note = D-Asp
  SITE 4: note = Azidolysine
  SITE 5: note = 3-amino-9-methoxy-2,6,8-trimethyl-10-phenyl-deca-4,6-dienoic acid
  SITE 6: note = D-Glu
  SITE 7: note = N-methyldehydroalanine
  CROSSLNK 1..7: note = peptide bond
ALDKXEX

SEQ ID NO: 9 - protein, 7 aa, synthetic construct
  SITE 1: note = D-Ala
  SITE 3: note = D-Asp
  SITE 4: note = Orn
  SITE 5: note = 3-amino-9-methoxy-2,6,8-trimethyl-10-phenyl-deca-4,6-dienoic acid
  SITE 6: note = D-Glu
  SITE 7: note = N-methyldehydroalanine
  CROSSLNK 1..7: note = Peptide bond
ALDXXEX

SEQ ID NO: 10 - protein, 7 aa, synthetic construct
  SITE 1: note = D-Ala
  SITE 3: note = D-Asp
  SITE 4: note = Propargyllysine
  SITE 5: note = 3-amino-9-methoxy-2,6,8-trimethyl-10-phenyl-deca-4,6-dienoic acid
  SITE 6: note = D-Glu
  SITE 7: note = N-methyldehydroalanine
  CROSSLNK 1..7: note = Peptide bond
ALDKXEX

SEQ ID NO: 11 - protein, 7 aa, synthetic construct
  SITE 1: note = D-Azidoalanine
  SITE 3: note = D-Asp
  SITE 5: note = 3-amino-9-methoxy-2,6,8-trimethyl-10-phenyl-deca-4,6-dienoic acid
  SITE 6: note = D-Glu
  SITE 7: note = N-methyldehydroalanine
  CROSSLNK 1..7: note = Peptide bond
AWDRXEX

SEQ ID NO: 12 - protein, 7 aa, synthetic construct
  SITE 1: note = D-Ala
  SITE 3: note = D-Asp
  SITE 5: note = 3-amino-9-methoxy-2,6,8-trimethyl-10-phenyl-deca-4,6-dienoic acid
  SITE 6: note = D-Glu
  SITE 7: note = Azidoproline-MDap
  CROSSLNK 1..7: note = Peptide bond
ALDRXEX

SEQ ID NO: 13 - protein, 7 aa, synthetic construct
  SITE 1: note = D-Ala
  SITE 3: note = D-Asp
  SITE 4: note = Azidonorvaline
  SITE 5: note = 3-amino-9-methoxy-2,6,8-trimethyl-10-phenyl-deca-4,6-dienoic acid
  SITE 6: note = D-Glu
  SITE 7: note = N-methyldehydroalanine
  CROSSLNK 1..7: note = Peptide bond
AYDXXEX

SEQ ID NO: 14 - protein, 8 aa, synthetic construct
  SITE 2: note = 6-(2-aminoethoxy)tryptophan
  CROSSLNK 1..8: note = Peptide bond
  CROSSLNK 2..6: note = Sulfoxide bridge
  SITE 1: note = dihydroxyisoleucine
  SITE 8: note = hydroxyproline
IWGCGCNP

SEQ ID NO: 15 - protein, 8 aa, synthetic construct
  SITE 1: note = 4,5-[(oxycarbonyl)-propargylamine]-dihydroxyisoleucine
  CROSSLNK 1..8: note = Peptide bond
  CROSSLNK 2..6: note = Sulfoxide bridge
  SITE 8: note = hydroxyproline
IWGCGCNP

SEQ ID NO: 16 - protein, 7 aa, Microcystis sp.
  SITE 1: note = D-Ala
  SITE 3: note = D-Asp
  SITE 5: note = 3-amino-9-methoxy-2,6,8-trimethyl-10-phenyl-deca-4,6-dienoic acid
  SITE 6: note = D-Glu
  SITE 7: note = N-methyldehydroalanine
  CROSSLNK 1..7: note = Peptide bond
ALDRXEX